European Patent Specification EP 3 139 955 B1, published March 20, 2024. Title: FUSION PROTEINS FOR TREATING CANCER AND RELATED METHODS. Applicant: President and Fellows of Harvard College Dana Farber Cancer Instititute, Inc. The sequence listing filed with the application follows.

SEQUENCE LISTING (40 sequences)

SEQ ID NO: 1 - protein, 449 aa, Artificial Sequence
  Synthetic Polypeptide
EVQLVESGGGLVQPGGSLRLSCKVSGFTFSSYGMSWVRQAPGKGLEWVASISTGGYNTYYADSVKGRFTISRDNSKNTLYLQMNSLRAEDTAVYYCARGYSPYSYAMDYWGQGTTVTVSGGGGGSGGGGSGGGGSDIQMTQSPSSLSASVGDRVTITCRASTDIDNDMNWYQQKPGQAPKLLIYEGNSLQSGVPSRFSSSGSGTDFTLTISSLQPEDFATYYCLQSWNVPLTFGQGTKLEIKGEGGSGEGSSGEGSSSEGGGSEGGGSEGGGSEGGSCDLPQTHSLGSRRTLMLLAQMRRISPFSCLKDRHDFGFPQEEFDGNQFQKAQAISVLHEMIQQIFNLFSTKDSSAAWDETLLEKFYTELYQQLNDLEACVTQEVGVEETPLMNEDSILAVKKYFQRITLYLTEKKYSPCAWEVVRAEIMRSFSLSTNLQERLRRKEHHHHHH

SEQ ID NO: 2 - protein, 449 aa, Artificial Sequence
  Synthetic Polypeptide
EVQLVESGGGLVQPGGSLRLSCKVSGFTFSSYGMSWVRQAPGKGLEWVASISTGGYNTYYADSVKGRFTISRDNSKNTLYLQMNSLRAEDTAVYYCARGYSPYSYAMDYWGQGTTVTVSGGGGGSGGGGSGGGGSDIQMTQSPSSLSASVGDRVTITCRASTDIDNDMNWYQQKPGQAPKLLIYEGNSLQSGVPSRFSSSGSGTDFTLTISSLQPEDFATYYCLQSWNVPLTFGQGTKLEIKGEGGSGEGSSGEGSSSEGGGSEGGGSEGGGSEGGSCDLPQTHSLGSRRTLMLLAQMRRISPFSCAKDRHDFGFPQEEFDGNQFQKAQAISVLHEMIQQIFNLFSTKDSSAAWDETLLEKFYTELYQQLNDLEACVTQEVGVEETPLMNEDSILAVKKYFQRITLYLTEKKYSPCAWEVVRAEIMRSFSLSTNLQERLRRKEHHHHHH

SEQ ID NO: 3 - protein, 449 aa, Artificial Sequence
  Synthetic Polypeptide
EVQLVESGGGLVQPGGSLRLSCKVSGFTFSSYGMSWVRQAPGKGLEWVASISTGGYNTYYADSVKGRFTISRDNSKNTLYLQMNSLRAEDTAVYYCARGYSPYSYAMDYWGQGTTVTVSGGGGGSGGGGSGGGGSDIQMTQSPSSLSASVGDRVTITCRASTDIDNDMNWYQQKPGQAPKLLIYEGNSLQSGVPSRFSSSGSGTDFTLTISSLQPEDFATYYCLQSWNVPLTFGQGTKLEIKGEGGSGEGSSGEGSSSEGGGSEGGGSEGGGSEGGSCDLPQTHSLGSRRTLMLLAQMRRISPFSCLKDRHDFGFPQEEFDGNQFQKAQAISVLHEMIQQIFNLFSTKDSSAAWDETLLEKFYTELYQQLNDLEACVTQEVGVEETPLMNEDSILAVKKYFQRITLYLTEKKYSPCAWEVVAAEIMRSFSLSTNLQERLRRKEHHHHHH

SEQ ID NO: 4 - protein, 449 aa, Artificial Sequence
  Synthetic Polypeptide
EVQLVESGGGLVQPGGSLRLSCKVSGFTFSSYGMSWVRQAPGKGLEWVASISTGGYNTYYADSVKGRFTISRDNSKNTLYLQMNSLRAEDTAVYYCARGYSPYSYAMDYWGQGTTVTVSGGGGGSGGGGSGGGGSDIQMTQSPSSLSASVGDRVTITCRASTDIDNDMNWYQQKPGQAPKLLIYEGNSLQSGVPSRFSSSGSGTDFTLTISSLQPEDFATYYCLQSWNVPLTFGQGTKLEIKGEGGSGEGSSGEGSSSEGGGSEGGGSEGGGSEGGSCDLPQTHSLGSRRTLMLLAQMRRISPFSCLKDRHDFGFPQEEFDGNQFQKAQAISVLHAMIQQIFNLFSTKDSSAAWDETLLEKFYTELYQQLNDLEACVTQEVGVEETPLMNEDSILAVKKYFQRITLYLTEKKYSPCAWEVVRAEIARSFSLSTNLQERLRRKEHHHHHH

SEQ ID NO: 5 - protein, 449 aa, Artificial Sequence
  Synthetic Polypeptide
EVQLVESGGGLVQPGGSLRLSCKVSGFTFSSYGMSWVRQAPGKGLEWVASISTGGYNTYYADSVKGRFTISRDNSKNTLYLQMNSLRAEDTAVYYCARGYSPYSYAMDYWGQGTTVTVSGGGGGSGGGGSGGGGSDIQMTQSPSSLSASVGDRVTITCRASTDIDNDMNWYQQKPGQAPKLLIYEGNSLQSGVPSRFSSSGSGTDFTLTISSLQPEDFATYYCLQSWNVPLTFGQGTKLEIKGEGGSGEGSSGEGSSSEGGGSEGGGSEGGGSEGGSCDLPQTHSLGSRRTLMLLAQMRRISPFSCLKDRHDFGFPQEEFDGNQFQKAQAISVLAEMIQQIFNLFSTKDSSAAWDETLLEKFYTELYQQLNDLEACVTQEVGVEETPLMNEDSILAVKKYFQRITLYLTEKKYSPCAWEVVRAEIMASFSLSTNLQERLRRKEHHHHHH

SEQ ID NO: 6 - DNA, 1350 bp, Artificial Sequence
  Synthetic Polynucleotide
gaagttcaattggttgagtctggtggaggtttggttcaaccaggaggttccttgagattgtcatgtaaagtttctggttttactttctcttcctatggaatgtcttgggttagacaagctcctggaaagggtttggaatgggttgcttccatctcaaccggtggttacaacacatattacgctgattccgttaaaggtagattcactatctccagagataactctaagaacactttgtatttgcaaatgaactctttgagagctgaagatactgctgtttactattgtgcgcgcggttactctccatattcttacgctatggattattggggtcaaggtactactgttactgtttctggtggaggtggaggttcaggaggtggaggaagtggaggaggtggatcagacatccagatgacacaatcaccatcttccttgtcagcttctgttggagatagagttactattacatgtagagcttccactgacatcgataacgacatgaattggtatcagcaaaaacctggacaggcgccaaagttgttgatctacgagggtaactcattgcaatctggagttccttccagattttcatcttccggttccggaacagatttcactttgacaatctcttccttgcagccagaagactttgctacttattactgtttgcaatcatggaatgttcctttgacattcggtcaaggaactaaattggagattaagggtgaaggagggtcaggtgaaggttcctccggtgagggttcctcatccgaagggggaggatctgaaggcggtggctctgagggtggaggttcagagggagggtcatgtgacttgcctcaaactcattctttgggttctagaagaactttgatgttgttggctcaaatgagaagaatctctcctttctcttgtttgaaggacagacatgacttcggtttccctcaagaggagttcgacggtaaccaattccaaaaggctcaagctatctctgtcttgcatgagatgatccaacaaatcttcaacttgttctctactaaggactcttctgctgcttgggacgagactttgttggagaagttctacactgagttgtaccaacaattgaacgacttggaggcttgtgtcactcaagaggtcggtgtcgaggagactcctttgatgaacgaggactctatcttggctgtcaagaagtacttccaaagaatcactttgtacttgactgagaagaagtactctccttgtgcttgggaggtcgtcagagctgagatcatgagatctttctctttgtctactaacttgcaagagagattgagaagaaaggagcatcaccatcaccatcactaa

SEQ ID NO: 7 - DNA, 1350 bp, Artificial Sequence
  Synthetic Polynucleotide
gaagttcaattggttgagtctggtggaggtttggttcaaccaggaggttccttgagattgtcatgtaaagtttctggttttactttctcttcctatggaatgtcttgggttagacaagctcctggaaagggtttggaatgggttgcttccatctcaaccggtggttacaacacatattacgctgattccgttaaaggtagattcactatctccagagataactctaagaacactttgtatttgcaaatgaactctttgagagctgaagatactgctgtttactattgtgcgcgcggttactctccatattcttacgctatggattattggggtcaaggtactactgttactgtttctggtggaggtggaggttcaggaggtggaggaagtggaggaggtggatcagacatccagatgacacaatcaccatcttccttgtcagcttctgttggagatagagttactattacatgtagagcttccactgacatcgataacgacatgaattggtatcagcaaaaacctggacaggcgccaaagttgttgatctacgagggtaactcattgcaatctggagttccttccagattttcatcttccggttccggaacagatttcactttgacaatctcttccttgcagccagaagactttgctacttattactgtttgcaatcatggaatgttcctttgacattcggtcaaggaactaaattggagattaagggtgaaggagggtcaggtgaaggttcctccggtgagggttcctcatccgaagggggaggatctgaaggcggtggctctgagggtggaggttcagagggagggtcatgtgacttgcctcaaactcattctttgggttctagaagaactttgatgttgttggctcaaatgagaagaatctctcctttctcttgtgctaaggacagacatgacttcggtttccctcaagaggagttcgacggtaaccaattccaaaaggctcaagctatctctgtcttgcatgagatgatccaacaaatcttcaacttgttctctactaaggactcttctgctgcttgggacgagactttgttggagaagttctacactgagttgtaccaacaattgaacgacttggaggcttgtgtcactcaagaggtcggtgtcgaggagactcctttgatgaacgaggactctatcttggctgtcaagaagtacttccaaagaatcactttgtacttgactgagaagaagtactctccttgtgcttgggaggtcgtcagagctgagatcatgagatctttctctttgtctactaacttgcaagagagattgagaagaaaggagcatcaccatcaccatcactaa

SEQ ID NO: 8 - DNA, 1350 bp, Artificial Sequence
  Synthetic Polynucleotide
gaagttcaattggttgagtctggtggaggtttggttcaaccaggaggttccttgagattgtcatgtaaagtttctggttttactttctcttcctatggaatgtcttgggttagacaagctcctggaaagggtttggaatgggttgcttccatctcaaccggtggttacaacacatattacgctgattccgttaaaggtagattcactatctccagagataactctaagaacactttgtatttgcaaatgaactctttgagagctgaagatactgctgtttactattgtgcgcgcggttactctccatattcttacgctatggattattggggtcaaggtactactgttactgtttctggtggaggtggaggttcaggaggtggaggaagtggaggaggtggatcagacatccagatgacacaatcaccatcttccttgtcagcttctgttggagatagagttactattacatgtagagcttccactgacatcgataacgacatgaattggtatcagcaaaaacctggacaggcgccaaagttgttgatctacgagggtaactcattgcaatctggagttccttccagattttcatcttccggttccggaacagatttcactttgacaatctcttccttgcagccagaagactttgctacttattactgtttgcaatcatggaatgttcctttgacattcggtcaaggaactaaattggagattaagggtgaaggagggtcaggtgaaggttcctccggtgagggttcctcatccgaagggggaggatctgaaggcggtggctctgagggtggaggttcagagggagggtcatgtgacttgcctcaaactcattctttgggttctagaagaactttgatgttgttggctcaaatgagaagaatctctcctttctcttgtttgaaggacagacatgacttcggtttccctcaagaggagttcgacggtaaccaattccaaaaggctcaagctatctctgtcttgcatgagatgatccaacaaatcttcaacttgttctctactaaggactcttctgctgcttgggacgagactttgttggagaagttctacactgagttgtaccaacaattgaacgacttggaggcttgtgtcactcaagaggtcggtgtcgaggagactcctttgatgaacgaggactctatcttggctgtcaagaagtacttccaaagaatcactttgtacttgactgagaagaagtactctccttgtgcttgggaggtcgtcgctgctgagatcatgagatctttctctttgtctactaacttgcaagagagattgagaagaaaggagcatcaccatcaccatcactaa

SEQ ID NO: 9 - DNA, 1350 bp, Artificial Sequence
  Synthetic Polynucleotide
gaagttcaattggttgagtctggtggaggtttggttcaaccaggaggttccttgagattgtcatgtaaagtttctggttttactttctcttcctatggaatgtcttgggttagacaagctcctggaaagggtttggaatgggttgcttccatctcaaccggtggttacaacacatattacgctgattccgttaaaggtagattcactatctccagagataactctaagaacactttgtatttgcaaatgaactctttgagagctgaagatactgctgtttactattgtgcgcgcggttactctccatattcttacgctatggattattggggtcaaggtactactgttactgtttctggtggaggtggaggttcaggaggtggaggaagtggaggaggtggatcagacatccagatgacacaatcaccatcttccttgtcagcttctgttggagatagagttactattacatgtagagcttccactgacatcgataacgacatgaattggtatcagcaaaaacctggacaggcgccaaagttgttgatctacgagggtaactcattgcaatctggagttccttccagattttcatcttccggttccggaacagatttcactttgacaatctcttccttgcagccagaagactttgctacttattactgtttgcaatcatggaatgttcctttgacattcggtcaaggaactaaattggagattaagggtgaaggagggtcaggtgaaggttcctccggtgagggttcctcatccgaagggggaggatctgaaggcggtggctctgagggtggaggttcagagggagggtcatgtgacttgcctcaaactcattctttgggttctagaagaactttgatgttgttggctcaaatgagaagaatctctcctttctcttgtttgaaggacagacatgacttcggtttccctcaagaggagttcgacggtaaccaattccaaaaggctcaagctatctctgtcttgcatgcgatgatccaacaaatcttcaacttgttctctactaaggactcttctgctgcttgggacgagactttgttggagaagttctacactgagttgtaccaacaattgaacgacttggaggcttgtgtcactcaagaggtcggtgtcgaggagactcctttgatgaacgaggactctatcttggctgtcaagaagtacttccaaagaatcactttgtacttgactgagaagaagtactctccttgtgcttgggaggtcgtcagagctgagatcgcgagatctttctctttgtctactaacttgcaagagagattgagaagaaaggagcatcaccatcaccatcactaa

SEQ ID NO: 10 - DNA, 1350 bp, Artificial Sequence
  Synthetic Polynucleotide
gaagttcaattggttgagtctggtggaggtttggttcaaccaggaggttccttgagattgtcatgtaaagtttctggttttactttctcttcctatggaatgtcttgggttagacaagctcctggaaagggtttggaatgggttgcttccatctcaaccggtggttacaacacatattacgctgattccgttaaaggtagattcactatctccagagataactctaagaacactttgtatttgcaaatgaactctttgagagctgaagatactgctgtttactattgtgcgcgcggttactctccatattcttacgctatggattattggggtcaaggtactactgttactgtttctggtggaggtggaggttcaggaggtggaggaagtggaggaggtggatcagacatccagatgacacaatcaccatcttccttgtcagcttctgttggagatagagttactattacatgtagagcttccactgacatcgataacgacatgaattggtatcagcaaaaacctggacaggcgccaaagttgttgatctacgagggtaactcattgcaatctggagttccttccagattttcatcttccggttccggaacagatttcactttgacaatctcttccttgcagccagaagactttgctacttattactgtttgcaatcatggaatgttcctttgacattcggtcaaggaactaaattggagattaagggtgaaggagggtcaggtgaaggttcctccggtgagggttcctcatccgaagggggaggatctgaaggcggtggctctgagggtggaggttcagagggagggtcatgtgacttgcctcaaactcattctttgggttctagaagaactttgatgttgttggctcaaatgagaagaatctctcctttctcttgtttgaaggacagacatgacttcggtttccctcaagaggagttcgacggtaaccaattccaaaaggctcaagctatctctgtcttggctgagatgatccaacaaatcttcaacttgttctctactaaggactcttctgctgcttgggacgagactttgttggagaagttctacactgagttgtaccaacaattgaacgacttggaggcttgtgtcactcaagaggtcggtgtcgaggagactcctttgatgaacgaggactctatcttggctgtcaagaagtacttccaaagaatcactttgtacttgactgagaagaagtactctccttgtgcttgggaggtcgtcagagctgagatcatggcatctttctctttgtctactaacttgcaagagagattgagaagaaaggagcatcaccatcaccatcactaa

SEQ ID NO: 11 - protein, 5 aa, Artificial Sequence
  Synthetic Polypeptide
GGGSE

SEQ ID NO: 12 - protein, 5 aa, Artificial Sequence
  Synthetic Polypeptide
GSESG

SEQ ID NO: 13 - protein, 5 aa, Artificial Sequence
  Synthetic Polypeptide
GSEGS

SEQ ID NO: 14 - protein, 35 aa, Artificial Sequence
  Synthetic Polypeptide
GEGGSGEGSSGEGSSSEGGGSEGGGSEGGGSEGGS

SEQ ID NO: 15 - protein, 119 aa, Artificial Sequence
  Synthetic Polypeptide
EVQLVESGGGLVQPGGSLRLSCKVSGFTFSSYGMSWVRQAPGKGLEWVASISTGGYNTYYADSVKGRFTISRDNSKNTLYLQMNSLRAEDTAVYYCARGYSPYSYAMDYWGQGTTVTVS

SEQ ID NO: 16 - protein, 107 aa, Artificial Sequence
  Synthetic Polypeptide
DIQMTQSPSSLSASVGDRVTITCRASTDIDNDMNWYQQKPGQAPKLLIYEGNSLQSGVPSRFSSSGSGTDFTLTISSLQPEDFATYYCLQSWNVPLTFGQGTKLEIK

SEQ ID NO: 17 - protein, 9 aa, Artificial Sequence
  Synthetic Polypeptide
KGNYVVTDH

SEQ ID NO: 18 - protein, 166 aa, Artificial Sequence
  Synthetic Polypeptide
CDLPQTHSLGSRRTLMLLAQMRRISPFSCLKDRHDFGFPQEEFDGNQFQKAQAISVLHEMIQQIFNLFSTKDSSAAWDETLLEKFYTELYQQLNDLEACVTQEVGVEETPLMNEDSILAVKKYFQRITLYLTEKKYSPCAWEVVRAEIMRSFSLSTNLQERLRRKE

SEQ ID NO: 19 - DNA, 15 bp, Artificial Sequence
  Synthetic Polynucleotide
agagaggctgaagct

SEQ ID NO: 20 - protein, 5 aa, Artificial Sequence
  Synthetic Polypeptide
REAEA

SEQ ID NO: 21 - DNA, 21 bp, Artificial Sequence
  Synthetic Polynucleotide
catcaccatcaccatcactaa

SEQ ID NO: 22 - DNA, 10 bp, Artificial Sequence
  Synthetic Polynucleotide
gtttgtagcc

SEQ ID NO: 23 - protein, 6 aa, Artificial Sequence
  Synthetic Polypeptide
EEFGNQ

SEQ ID NO: 24 - protein, 7 aa, Artificial Sequence
  Synthetic Polypeptide
EEFDGNQ

SEQ ID NO: 25 - protein, 5 aa, Artificial Sequence
  Synthetic Polypeptide
GEGGS

SEQ ID NO: 26 - DNA, 105 bp, Artificial Sequence
  Synthetic Polynucleotide
ggtgaaggagggtcaggtgaaggttcctccggtgagggttcctcatccgaagggggaggatctgaaggcggtggctctgagggtggaggttcagagggagggtca

SEQ ID NO: 27 - protein, 35 aa, Artificial Sequence
  Synthetic Polypeptide
GEGGSEGGSEGSGESSGEGGSEGSGESGGESGGES

SEQ ID NO: 28 - DNA, 105 bp, Artificial Sequence
  Synthetic Polynucleotide
ggtgaaggagggtcagaaggaggttccgagggttctggtgaatcatccggagaaggaggatctgaaggctcaggcgagtctggtggagagtcagggggagagtca

SEQ ID NO: 29 - protein, 166 aa, Artificial Sequence
  Synthetic Polypeptide
CDLPQTHSLGNRRALILLAQMRRISPFSCLKDRHDFEFPQEEFDDKQFQKAQAISVLHEMIQQTFNLFSTKDSSAALDETLLDEFYIELDQQLNDLESCVMQEVGVIESPLMYEDSILAVRKYFQRITLYLTEKKYSSCAWEVVRAEIMRSFSLSINLQKRLKSKE

SEQ ID NO: 30 - protein, 165 aa, Homo sapiens
CDLPQTHSLGSRRTLMLLAQMRKISLFSCLKDRHDFGFPQEEFGNQFQKAETIPVLHEMIQQIFNLFSTKDSSAAWDETLLDKFYTELYQQLNDLEACVIQGVGVTETPLMKEDSILAVRKYFQRITLYLKEKKYSPCAWEVVRAEIMRSFSLSTNLQESLRSKE

SEQ ID NO: 31 - protein, 166 aa, Homo sapiens
CDLPETHSLDNRRTLMLLAQMSRISPSSCLMDRHDFGFPQEEFDGNQFQKAPAISVLHELIQQIFNLFTTKDSSAAWDEDLLDKFCTELYQQLNDLEACVMQEERVGETPLMNADSILAVKKYFRRITLYLTEKKYSPCAWEVVRAEIMRSLSLSTNLQERLRRKE

SEQ ID NO: 32 - protein, 166 aa, Homo sapiens
CDLPQTHSLSNRRTLMIMAQMGRISPFSCLKDRHDFGFPQEEFDGNQFQKAQAISVLHEMIQQTFNLFSTKDSSATWDETLLDKFYTELYQQLNDLEACMMQEVGVEDTPLMNVDSILTVRKYFQRITLYLTEKKYSPCAWEVVRAEIMRSFSLSANLQERLRRKE

SEQ ID NO: 33 - protein, 166 aa, Homo sapiens
CDLPQTHSLGNRRALILLAQMGRISPFSCLKDRHDFGFPQEEFDGNQFQKAQAISVLHEMIQQTFNLFSTKDSSATWEQSLLEKFSTELNQQLNDLEACVIQEVGVEETPLMNVDSILAVKKYFQRITLYLTEKKYSPCAWEVVRAEIMRSFSLSKIFQERLRRKE

SEQ ID NO: 34 - protein, 166 aa, Homo sapiens
CDLPQTHSLGNRRALILLAQMGRISHFSCLKDRHDFGFPEEEFDGHQFQKAQAISVLHEMIQQTFNLFSTEDSSAAWEQSLLEKFSTELYQQLNDLEACVIQEVGVEETPLMNEDSILAVRKYFQRITLYLTEKKYSPCAWEVVRAEIMRSLSFSTNLQKRLRRKD

SEQ ID NO: 35 - protein, 166 aa, Homo sapiens
CDLPQTHSLGNRRALILLAQMGRISPFSCLKDRHDFGLPQEEFDGNQFQKTQAISVLHEMIQQTFNLFSTEDSSAAWEQSLLEKFSTELYQQLNNLEACVIQEVGMEETPLMNEDSILAVRKYFQRITLYLTEKKYSPCAWEVVRAEIMRSLSFSTNLQKRLRRKD

SEQ ID NO: 36 - protein, 166 aa, Homo sapiens
CDLPQTHSLGHRRTMMLLAQMRRISLFSCLKDRHDFRFPQEEFDGNQFQKAEAISVLHEVIQQTFNLFSTKDSSVAWDERLLDKLYTELYQQLNDLEACVMQEVWVGGTPLMNEDSILAVRKYFQRITLYLTEKKYSPCAWEVVRAEIMRSFSSSRNLQERLRRKE

SEQ ID NO: 37 - protein, 166 aa, Homo sapiens
CNLSQTHSLNNRRTLMLMAQMRRISPFSCLKDRHDFEFPQEEFDGNQFQKAQAISVLHEMMQQTFNLFSTKNSSAAWDETLLEKFYIELFQQMNDLEACVIQEVGVEETPLMNEDSILAVKKYFQRITLYLMEKKYSPCAWEVVRAEIMRSLSFSTNLQKRLRRKD

SEQ ID NO: 38 - protein, 166 aa, Homo sapiens
CDLPQTHSLGNRRALILLGQMGRISPFSCLKDRHDFRIPQEEFDGNQFQKAQAISVLHEMIQQTFNLFSTEDSSAAWEQSLLEKFSTELYQQLNDLEACVIQEVGVEETPLMNEDSILAVRKYFQRITLYLIERKYSPCAWEVVRAEIMRSLSFSTNLQKRLRRKD

SEQ ID NO: 39 - protein, 165 aa, Homo sapiens
CDLPQTHSLGSRRTLMLLAQMRRISLFSCLKDRHDFGFPQEEFGNQFQKAETIPVLHEMIQQIFNLFSTKDSSAAWDETLLDKFYTELYQQLNDLEACVIQGVGVTETPLMNEDSILAVRKYFQRITLYLKEKKYSPCAWEVVRAEIMRSFSLSTNLQESLRSKE

SEQ ID NO: 40 - protein, 166 aa, Homo sapiens
CDLPQTHSLGNRRALILLAQMGRISHFSCLKDRYDFGFPQEVFDGNQFQKAQAISAFHEMIQQTFNLFSTKDSSAAWDETLLDKFYIELFQQLNDLEACVTQEVGVEEIALMNEDSILAVRKYFQRITLYLMGKKYSPCAWEVVRAEIMRSFSFSTNLQKGLRRKD